European Patent Application EP 4 692 119 A1, published February 11, 2026. Title: ANTIBODY OR ANTIGEN-BINDING FRAGMENT THEREOF TARGETING CD3 AND USE THEREOF. Applicant: SANYOU BIOPHARMACEUTICALS CO., LTD. Application WO. The sequence listing filed with the application follows.

SEQUENCE LISTING (81 sequences)

SEQ ID NO: 1 - protein, 125 aa, synthetic construct
EVQLVESGGGLVQPGGSLKLSCAASGFTFNKYAMNWVRQAPGKGLEWVARIRSKYNNYATYYADSVKDRFTISRDDSKNTAYLQMNNLKTEDTAVYYCVRHGNFGNSYISYWAYWGQGTLVTVSS

SEQ ID NO: 2 - protein, 109 aa, synthetic construct
QTVVTQEPSLTVSPGGTVTLTCGSSTGAVTSGYYPNWVQQKPGQAPRGLIGGTKFLAPGTPARFSGSLLGGKAALTLSGVQPEDEAEYYCALWYSNRWVFGGGTKLTVL

SEQ ID NO: 3 - protein, 27 aa, synthetic construct
QDGNEEMGGITQTPYKVSISGTTVILT

SEQ ID NO: 4 - protein, 225 aa, synthetic construct
THTCPPCPAPELLGGPSVFLFPPKPKDTLMISRTPEVTCVVVDVSHEDPQVKFNWYVDGVQVHNAKTKPREQQYNSTYRVVSVLTVLHQNWLDGKEYKCKVSNKALPAPIEKTISKAKGQPREPQVYTLPPSREEMTKNQVSLTCLVKGFYPSDIAVEWESNGQPENNYKTTPPVLDSDGSFFLYSKLTVDKSRWQQGNVFSCSVMHEALHNHYTQKSLSLSPGK

SEQ ID NO: 5 - protein, 171 aa, synthetic construct
MEHSTFLSGLVLATLLSQVSPFKIPIEELEDRVFVNCNTSITWVEGTVGTLLSDITRLDLGKRILDPRGIYRCNGTDIYKDKESTVQVHYRMCQSCVELDPATVAGIIVTDVIATLLLALGVFCFAGHETGRLSGAADTQALLRNDQVYQPLRDRDDAQYSHLGGNWARNK

SEQ ID NO: 6 - protein, 207 aa, synthetic construct
MQSGTHWRVLGLCLLSVGVWGQDGNEEMGGITQTPYKVSISGTTVILTCPQYPGSEILWQHNDKNIGGDEDDKNIGSDEDHLSLKEFSELEQSGYYVCYPRGSKPEDANFYLYLRARVCENCMEMDVMSVATIVIVDICITGGLLLLVYYWSKNRKAKAKPVTRGAGAGGRQRGQNKERPPPVPNPDYEPIRKGQRDLYSGLNQRRI

SEQ ID NO: 7 - protein, 249 aa, synthetic construct
QTVVTQEPSLTVSPGGTVTLTCGSSTGAVTSGYYPNWVQQKPGQAPRGLIGGTKFLAPGTPARFSGSLLGGKAALTLSGVQPEDEAEYYCALWYSNRWVFGGGTKLTVLGGGGSGGGGSGGGGSEVQLVESGGGLVQPGGSLKLSCAASGFTFNKYAMNWVRQAPGKGLEWVARIRSKYNNYATYYADSVKDRFTISRDDSKNTAYLQMNNLKTEDTAVYYCVRHGNFGNSYISYWAYWGQGTLVTVSS

SEQ ID NO: 8 - protein, 249 aa, synthetic construct
QTVVTQEPSLTVSPGGTVTLTCGSSTGAVTSGYYPNWVQQKPGQAPRALIYGTKFLAPGTPARFSGSLLGGKAALTLSGVQPEDEAEYYCALWYSNRWVFGGGTKLTVLGGGGSGGGGSGGGGSEVQLVESGGGLVQPGGSLKLSCAASGFTFNKYAMNWVRQAPGKGLEWVGRIRSKYNNYATYYADSVKDRFTISRDDSKNTAYLQMNNLKTEDTAVYYCVRHGNFGNSYISYWAYWGQGTTVTVSS

SEQ ID NO: 9 - protein, 249 aa, synthetic construct
QTVVTQEPSLTVSPGGTVTLTCGSSTGAVTSGYYPNWVQQKPGQAPRALIGGTKFLAPGTPARFSGSLLGGKAALTLSGVQPEDEAEYYCALWYSNRWVFGGGTKLTVLGGGGSGGGGSGGGGSEVQLVESGGGLVQPGGSLKLSCAASGFTFSKYAMNWVRQAPGKGLEWVARIRSKYNNYATYYADSVKDRFTISRDDSKNTAYLQMNNLKTEDTAVYYCVRHGNFGNSYISYWAYWGQGTTVTVSS

SEQ ID NO: 10 - protein, 249 aa, synthetic construct
QTVVTQEPSLTVSPGGTVTLTCGSSTGAVTSGYYPNWVQQKPGQAPRGLIGGTKFLAPGTPARFSGSLLGGKAALTLSGVQPEDEAEYYCALWYSNRWVFGGGTKLTVLGGGGSGGGGSGGGGSEVQLVESGGGLVQPGGSLKLSCAASGFTFSKYAMNWVRQASGKGLEWVGRIRSKYNNYATYYADSVKDRFTISRDDSKNTAYLQMNNLKTEDTAVYYCVRHGNFGNSYISYWAYWGQGTTVTVSS

SEQ ID NO: 11 - protein, 249 aa, synthetic construct
QTVVTQEPSLTVSPGGTVTLTCGSSTGAVTSGYYPNWVQQKPGQAPRGLIGGTKFLAPGTPARFSGSLLGGKAALTLSGVQPEDEAEYYCALWVDNRWVFGGGTKLTVLGGGGSGGGGSGGGGSEVQLVESGGGLVQPGGSLKLSCAASGFTFNKYAMNWVRQAPGKGLEWVARIRSKYNNYATYYADSVKDRFTISRDDSKNTAYLQMNNLKTEDTAVYYCVRHGNFGNSYISYWAYWGQGTLVTVSS

SEQ ID NO: 12 - protein, 249 aa, synthetic construct
QTVVTQEPSLTVSPGGTVTLTCGSSTGAVTSGYYPNWVQQKPGQAPRGLIGGTHFLAPGTPARFSGSLLGGKAALTLSGVQPEDEAEYYCALWYSNRWVFGGGTKLTVLGGGGSGGGGSGGGGSEVQLVESGGGLVQPGGSLKLSCAASGFTFPKYAMNWVRQAPGKGLEWVARIRSKYNNYETYYADSVKDRFTISRDDSKNTAYLQMNNLKTEDTAVYYCVRHGNFGNSYISYWAYWGQGTLVTVSS

SEQ ID NO: 13 - protein, 249 aa, synthetic construct
QTVVTQEPSLTVSPGGTVTLTCGSSTGAVTSGYYPNWVQQKPGQAPRGLIGGTKFLAPGTPARFSGSLLGGKAALTLSGVQPEDEAEYYCALWQENRWVFGGGTKLTVLGGGGSGGGGSGGGGSEVQLVESGGGLVQPGGSLKLSCAASGFTFNKYAMNWVRQAPGKGLEWVARIRSKYNNYATYYADSVKDRFTISRDDSKNTAYLQMNNLKTEDTAVYYCVRHGNFGNSYISYWAYWGQGTLVTVSS

SEQ ID NO: 14 - protein, 249 aa, synthetic construct
QTVVTQEPSLTVSPGGTVTLTCGSSTGAVTSGYYPNWVQQKPGQAPRALIYGTKFLAPGTPARFSGSLLGGKAALTLSGVQPEDEAEYYCALWYSNRWVFGGGTKLTVLGGGGSGGGGSGGGGSEVQLVESGGGLVQPGGSLKLSCAASGFTFSKYAMNWVRQASGKGLEWVGRIRSKYNNYATYYADSVKDRFTISRDDSKNTAYLQMNNLKTEDTAVYYCVRHGNFGNSYISYWAYWGQGTTVTVSS

SEQ ID NO: 15 - protein, 249 aa, synthetic construct
QTVVTQEPSLTVSPGGTVTLTCGSSTGAVTSGYYPNWVQQKPGQAPRALIGGTKFLAPGTPARFSGSLLGGKAALTLSGVQPEDEAEYYCALWYSNRWVFGGGTKLTVLGGGGSGGGGSGGGGSEVQLVESGGGLVQPGGSLKLSCAASGFTFSKYAMNWVRQAPGKGLEWVGRIRSKYNNYATYYADSVKDRFTISRDDSKNTAYLQMNNLKTEDTAVYYCVRHGNFGNSYISYWAYWGQGTTVTVSS

SEQ ID NO: 16 - protein, 249 aa, synthetic construct
QTVVTQEPSLTVSPGGTVTLTCGSSTGAVTSGYYPNWVQQKPGQAPRALIGGTKFLAPGTPARFSGSLLGGKAALTLSGVQPEDEAEYYCALWYSNRWVFGGGTKLTVLGGGGSGGGGSGGGGSEVQLVESGGGLVQPGGSLKLSCAASGFTFSKYAMNWVRQASGKGLEWVGRIRSKYNNYATYYADSVKDRFTISRDDSKNTAYLQMNNLKTEDTAVYYCVRHGNFGNSYISYWAYWGQGTTVTVSS

SEQ ID NO: 17 - protein, 249 aa, synthetic construct
QTVVTQEPSLTVSPGGTVTLTCGSSTGAVTSGYYPNWVQQKPGQAPRALIGGTKFLAPGTPARFSGSLLGGKAALTLSGVQPEDEAEYYCALWVDNRWVFGGGTKLTVLGGGGSGGGGSGGGGSEVQLVESGGGLVQPGGSLKLSCAASGFTFSKYAMNWVRQAPGKGLEWVARIRSKYNNYATYYADSVKDRFTISRDDSKNTAYLQMNNLKTEDTAVYYCVRHGNFGNSYISYWAYWGQGTTVTVSS

SEQ ID NO: 18 - protein, 249 aa, synthetic construct
QTVVTQEPSLTVSPGGTVTLTCGSSTGAVTSGYYPNWVQQKPGQAPRGLIGGTKFLAPGTPARFSGSLLGGKAALTLSGVQPEDEAEYYCALWVDNRWVFGGGTKLTVLGGGGSGGGGSGGGGSEVQLVESGGGLVQPGGSLKLSCAASGFTFSKYAMNWVRQASGKGLEWVGRIRSKYNNYATYYADSVKDRFTISRDDSKNTAYLQMNNLKTEDTAVYYCVRHGNFGNSYISYWAYWGQGTTVTVSS

SEQ ID NO: 19 - protein, 249 aa, synthetic construct
QTVVTQEPSLTVSPGGTVTLTCGSSTGAVTSGYYPNWVQQKPGQAPRALIYGTHFLAPGTPARFSGSLLGGKAALTLSGVQPEDEAEYYCALWYSNRWVFGGGTKLTVLGGGGSGGGGSGGGGSEVQLVESGGGLVQPGGSLKLSCAASGFTFPKYAMNWVRQAPGKGLEWVGRIRSKYNNYETYYADSVKDRFTISRDDSKNTAYLQMNNLKTEDTAVYYCVRHGNFGNSYISYWAYWGQGTTVTVSS

SEQ ID NO: 20 - protein, 249 aa, synthetic construct
QTVVTQEPSLTVSPGGTVTLTCGSSTGAVTSGYYPNWVQQKPGQAPRALIGGTHFLAPGTPARFSGSLLGGKAALTLSGVQPEDEAEYYCALWYSNRWVFGGGTKLTVLGGGGSGGGGSGGGGSEVQLVESGGGLVQPGGSLKLSCAASGFTFSKYAMNWVRQAPGKGLEWVARIRSKYNNYETYYADSVKDRFTISRDDSKNTAYLQMNNLKTEDTAVYYCVRHGNFGNSYISYWAYWGQGTTVTVSS

SEQ ID NO: 21 - protein, 249 aa, synthetic construct
QTVVTQEPSLTVSPGGTVTLTCGSSTGAVTSGYYPNWVQQKPGQAPRGLIGGTHFLAPGTPARFSGSLLGGKAALTLSGVQPEDEAEYYCALWYSNRWVFGGGTKLTVLGGGGSGGGGSGGGGSEVQLVESGGGLVQPGGSLKLSCAASGFTFSKYAMNWVRQASGKGLEWVGRIRSKYNNYETYYADSVKDRFTISRDDSKNTAYLQMNNLKTEDTAVYYCVRHGNFGNSYISYWAYWGQGTTVTVSS

SEQ ID NO: 22 - protein, 249 aa, synthetic construct
QTVVTQEPSLTVSPGGTVTLTCGSSTGAVTSGYYPNWVQQKPGQAPRALIYGTKFLAPGTPARFSGSLLGGKAALTLSGVQPEDEAEYYCALWQENRWVFGGGTKLTVLGGGGSGGGGSGGGGSEVQLVESGGGLVQPGGSLKLSCAASGFTFNKYAMNWVRQAPGKGLEWVGRIRSKYNNYATYYADSVKDRFTISRDDSKNTAYLQMNNLKTEDTAVYYCVRHGNFGNSYISYWAYWGQGTTVTVSS

SEQ ID NO: 23 - protein, 249 aa, synthetic construct
QTVVTQEPSLTVSPGGTVTLTCGSSTGAVTSGYYPNWVQQKPGQAPRALIGGTKFLAPGTPARFSGSLLGGKAALTLSGVQPEDEAEYYCALWQENRWVFGGGTKLTVLGGGGSGGGGSGGGGSEVQLVESGGGLVQPGGSLKLSCAASGFTFSKYAMNWVRQAPGKGLEWVARIRSKYNNYATYYADSVKDRFTISRDDSKNTAYLQMNNLKTEDTAVYYCVRHGNFGNSYISYWAYWGQGTTVTVSS

SEQ ID NO: 24 - protein, 249 aa, synthetic construct
QTVVTQEPSLTVSPGGTVTLTCGSSTGAVTSGYYPNWVQQKPGQAPRGLIGGTKFLAPGTPARFSGSLLGGKAALTLSGVQPEDEAEYYCALWQENRWVFGGGTKLTVLGGGGSGGGGSGGGGSEVQLVESGGGLVQPGGSLKLSCAASGFTFSKYAMNWVRQASGKGLEWVGRIRSKYNNYATYYADSVKDRFTISRDDSKNTAYLQMNNLKTEDTAVYYCVRHGNFGNSYISYWAYWGQGTTVTVSS

SEQ ID NO: 25 - protein, 229 aa, synthetic construct
ESKYGPPCPPCPAPEFLGGPSVFLFPPKPKDTLMISRTPEVTCVVVDVSQEDPEVQFNWYVDGVEVHNAKTKPREEQFNSTYRVVSVLTVLHQDWLNGKEYKCKVSNKGLPSSIEKTISKAKGQPREPQVYTLPPSQEEMTKNQVSLTCLVKGFYPSDIAVEWESNGQPENNYKTTPPVLDSDGSFFLYSRLTVDKSRWQEGNVFSCSVMHEALHNHYTQKSLSLSLGK

SEQ ID NO: 26 - protein, 125 aa, synthetic construct
EVQLVESGGGLVQPGGSLKLSCAASGFTFNKYAMNWVRQAPGKGLEWVGRIRSKYNNYATYYADSVKDRFTISRDDSKNTAYLQMNNLKTEDTAVYYCVRHGNFGNSYISYWAYWGQGTTVTVSS

SEQ ID NO: 27 - protein, 109 aa, synthetic construct
QTVVTQEPSLTVSPGGTVTLTCGSSTGAVTSGYYPNWVQQKPGQAPRALIYGTKFLAPGTPARFSGSLLGGKAALTLSGVQPEDEAEYYCALWYSNRWVFGGGTKLTVL

SEQ ID NO: 28 - protein, 125 aa, synthetic construct
EVQLVESGGGLVQPGGSLKLSCAASGFTFSKYAMNWVRQAPGKGLEWVARIRSKYNNYATYYADSVKDRFTISRDDSKNTAYLQMNNLKTEDTAVYYCVRHGNFGNSYISYWAYWGQGTTVTVSS

SEQ ID NO: 29 - protein, 109 aa, synthetic construct
QTVVTQEPSLTVSPGGTVTLTCGSSTGAVTSGYYPNWVQQKPGQAPRALIGGTKFLAPGTPARFSGSLLGGKAALTLSGVQPEDEAEYYCALWYSNRWVFGGGTKLTVL

SEQ ID NO: 30 - protein, 125 aa, synthetic construct
EVQLVESGGGLVQPGGSLKLSCAASGFTFSKYAMNWVRQASGKGLEWVGRIRSKYNNYATYYADSVKDRFTISRDDSKNTAYLQMNNLKTEDTAVYYCVRHGNFGNSYISYWAYWGQGTTVTVSS

SEQ ID NO: 31 - protein, 109 aa, synthetic construct
QTVVTQEPSLTVSPGGTVTLTCGSSTGAVTSGYYPNWVQQKPGQAPRGLIGGTKFLAPGTPARFSGSLLGGKAALTLSGVQPEDEAEYYCALWVDNRWVFGGGTKLTVL

SEQ ID NO: 32 - protein, 125 aa, synthetic construct
EVQLVESGGGLVQPGGSLKLSCAASGFTFPKYAMNWVRQAPGKGLEWVARIRSKYNNYETYYADSVKDRFTISRDDSKNTAYLQMNNLKTEDTAVYYCVRHGNFGNSYISYWAYWGQGTLVTVSS

SEQ ID NO: 33 - protein, 109 aa, synthetic construct
QTVVTQEPSLTVSPGGTVTLTCGSSTGAVTSGYYPNWVQQKPGQAPRGLIGGTHFLAPGTPARFSGSLLGGKAALTLSGVQPEDEAEYYCALWYSNRWVFGGGTKLTVL

SEQ ID NO: 34 - protein, 109 aa, synthetic construct
QTVVTQEPSLTVSPGGTVTLTCGSSTGAVTSGYYPNWVQQKPGQAPRGLIGGTKFLAPGTPARFSGSLLGGKAALTLSGVQPEDEAEYYCALWQENRWVFGGGTKLTVL

SEQ ID NO: 35 - protein, 125 aa, synthetic construct
EVQLVESGGGLVQPGGSLKLSCAASGFTFSKYAMNWVRQAPGKGLEWVGRIRSKYNNYATYYADSVKDRFTISRDDSKNTAYLQMNNLKTEDTAVYYCVRHGNFGNSYISYWAYWGQGTTVTVSS

SEQ ID NO: 36 - protein, 109 aa, synthetic construct
QTVVTQEPSLTVSPGGTVTLTCGSSTGAVTSGYYPNWVQQKPGQAPRALIGGTKFLAPGTPARFSGSLLGGKAALTLSGVQPEDEAEYYCALWVDNRWVFGGGTKLTVL

SEQ ID NO: 37 - protein, 125 aa, synthetic construct
EVQLVESGGGLVQPGGSLKLSCAASGFTFPKYAMNWVRQAPGKGLEWVGRIRSKYNNYETYYADSVKDRFTISRDDSKNTAYLQMNNLKTEDTAVYYCVRHGNFGNSYISYWAYWGQGTTVTVSS

SEQ ID NO: 38 - protein, 109 aa, synthetic construct
QTVVTQEPSLTVSPGGTVTLTCGSSTGAVTSGYYPNWVQQKPGQAPRALIYGTHFLAPGTPARFSGSLLGGKAALTLSGVQPEDEAEYYCALWYSNRWVFGGGTKLTVL

SEQ ID NO: 39 - protein, 125 aa, synthetic construct
EVQLVESGGGLVQPGGSLKLSCAASGFTFSKYAMNWVRQAPGKGLEWVARIRSKYNNYETYYADSVKDRFTISRDDSKNTAYLQMNNLKTEDTAVYYCVRHGNFGNSYISYWAYWGQGTTVTVSS

SEQ ID NO: 40 - protein, 109 aa, synthetic construct
QTVVTQEPSLTVSPGGTVTLTCGSSTGAVTSGYYPNWVQQKPGQAPRALIGGTHFLAPGTPARFSGSLLGGKAALTLSGVQPEDEAEYYCALWYSNRWVFGGGTKLTVL

SEQ ID NO: 41 - protein, 125 aa, synthetic construct
EVQLVESGGGLVQPGGSLKLSCAASGFTFSKYAMNWVRQASGKGLEWVGRIRSKYNNYETYYADSVKDRFTISRDDSKNTAYLQMNNLKTEDTAVYYCVRHGNFGNSYISYWAYWGQGTTVTVSS

SEQ ID NO: 42 - protein, 109 aa, synthetic construct
QTVVTQEPSLTVSPGGTVTLTCGSSTGAVTSGYYPNWVQQKPGQAPRALIYGTKFLAPGTPARFSGSLLGGKAALTLSGVQPEDEAEYYCALWQENRWVFGGGTKLTVL

SEQ ID NO: 43 - protein, 109 aa, synthetic construct
QTVVTQEPSLTVSPGGTVTLTCGSSTGAVTSGYYPNWVQQKPGQAPRALIGGTKFLAPGTPARFSGSLLGGKAALTLSGVQPEDEAEYYCALWQENRWVFGGGTKLTVL

SEQ ID NO: 44 - protein, 109 aa, synthetic construct; identical to SEQ ID NO: 34

SEQ ID NO: 45 - protein, 10 aa, synthetic construct
GFTFNKYAMN

SEQ ID NO: 46 - protein, 12 aa, synthetic construct
RIRSKYNNYATY

SEQ ID NO: 47 - protein, 14 aa, synthetic construct
HGNFGNSYISYWAY

SEQ ID NO: 48 - protein, 14 aa, synthetic construct
GSSTGAVTSGYYPN

SEQ ID NO: 49 - protein, 7 aa, synthetic construct
GTKFLAP

SEQ ID NO: 50 - protein, 9 aa, synthetic construct
ALWYSNRWV

SEQ ID NO: 51 - protein, 10 aa, synthetic construct
GFTFSKYAMN

SEQ ID NO: 52 - protein, 10 aa, synthetic construct
GFTFPKYAMN

SEQ ID NO: 53 - protein, 12 aa, synthetic construct
RIRSKYNNYETY

SEQ ID NO: 54 - protein, 7 aa, synthetic construct
GTHFLAP

SEQ ID NO: 55 - protein, 9 aa, synthetic construct
ALWVDNRWV

SEQ ID NO: 56 - protein, 9 aa, synthetic construct
ALWQENRWV

SEQ ID NO: 57 - protein, 25 aa, synthetic construct
EVQLVESGGGLVQPGGSLKLSCAAS

SEQ ID NO: 58 - protein, 14 aa, synthetic construct
WVRQAPGKGLEWVA

SEQ ID NO: 59 - protein, 39 aa, synthetic construct
YADSVKDRFTISRDDSKNTAYLQMNNLKTEDTAVYYCVR

SEQ ID NO: 60 - protein, 11 aa, synthetic construct
WGQGTLVTVSS

SEQ ID NO: 61 - protein, 22 aa, synthetic construct
QTVVTQEPSLTVSPGGTVTLTC

SEQ ID NO: 62 - protein, 15 aa, synthetic construct
WVQQKPGQAPRGLIG

SEQ ID NO: 63 - protein, 32 aa, synthetic construct
GTPARFSGSLLGGKAALTLSGVQPEDEAEYYC

SEQ ID NO: 64 - protein, 10 aa, synthetic construct
FGGGTKLTVL

SEQ ID NO: 65 - protein, 14 aa, synthetic construct
WVRQAPGKGLEWVG

SEQ ID NO: 66 - protein, 14 aa, synthetic construct
WVRQASGKGLEWVG

SEQ ID NO: 67 - protein, 11 aa, synthetic construct
WGQGTTVTVSS

SEQ ID NO: 68 - protein, 15 aa, synthetic construct
WVQQKPGQAPRALIY

SEQ ID NO: 69 - protein, 15 aa, synthetic construct
WVQQKPGQAPRALIG

SEQ ID NO: 70 - protein, 15 aa, synthetic construct
GGGGSGGGGSGGGGS

SEQ ID NO: 71 - protein, 249 aa, synthetic construct
QTVVTQEPSLTVSPGGTVTLTCGSSTGAVTSGYYPNWVQQKPGQAPRGLIGGTKFLAPGTPARFSGSLLGGKAALTLSGVQPEDEAEYYCALWYSNRWVFGGGTKLTVLGGGGSGGGGSGGGGSEVQLVESGGGLVQPGGSLKLSCAASGFTFSKYAMNWVRQAPGKGLEWVARIRSKYNNYATYYADSVKDRFTISRDDSKNTAYLQMNSLKTEDTAVYYCVRHGNFGNSYISYWAYWGQGTTVTVSS

SEQ ID NO: 72 - protein, 249 aa, synthetic construct
QTVVTQEPSLTVSPGGTVTLTCGSSTGAVTSGYYPNWVQQKPGQAPRGLIGGTKFLAPGTPARFSGSLLGGKAALTLSGVQPEDEAEYYCALWYSNRWVFGGGTKLTVLGGGGSGGGGSGGGGSEVQLVESGGGLVQPGGSLKLSCAASGFTFNKYAINWVRQAPGKGLEWVGRIRSKYNNYATYYADSVKDRFTISRDDSKNTAYLQMNSLKTEDTAVYYCTRHGNFGNSYISYWAYWGQGTTVTVSS

SEQ ID NO: 73 - protein, 249 aa, synthetic construct
QTVVTQEPSLTVSPGGTVTLTCGSSTGAVTSGYYPNWVQQKPGQAPRALIGGTKFLAPGTPARFSGSLLGGKAALTLSGVQPEDEAEYYCALWYSNRWVFGGGTKLTVLGGGGSGGGGSGGGGSEVQLVESGGGLVQPGGSLKLSCAASGFTFSKYAMNWVRQAPGKGLEWVARIRSKYNNYATYYADSVKDRFTISRDDSKNTAYLQMNNLKTEDTAVYYCTRHGNFGNSYISYWAYWGQGTTVTVSS

SEQ ID NO: 74 - protein, 249 aa, synthetic construct
QTVVTQEPSLTVSPGGTVTLTCGSSTGAVTSGYYPNWVQQKPGQAPRALIGGTKFLAPGTPARFSGSLLGGKAALTLSGVQPEDEAEYYCALWYSNRWVFGGGTKLTVLGGGGSGGGGSGGGGSEVQLVESGGGLVQPGGSLKLSCAASGFTFNKYAMNWVRQAPGKGLEWVARIRSKYNNYATYYADSVKDRFTISRDDSKNTAYLQMNSLKTEDTAVYYCVRHGNFGNSYISYWAYWGQGTTVTVSS

SEQ ID NO: 75 - protein, 249 aa, synthetic construct
QTVVTQEPSLTVSPGGTVTLTCGSSTGAVTSGYYPNWVQQKPGQAPRGLIGGTKFLAPGTPARFSGSLLGGKAALTLSGVQPEDEAEYYCALWYSDTWVFGGGTKLTVLGGGGSGGGGSGGGGSEVQLVESGGGLVQPGGSLKLSCAASGFTFNKYAMNWVRQAPGKGLEWVARIRSKYNNYATYYADSVKDRFTISRDDSKNTAYLQMNNLKTEDTAVYYCVRHGNFGNSYISYWAYWGQGTLVTVSS

SEQ ID NO: 76 - protein, 249 aa, synthetic construct
QTVVTQEPSLTVSPGGTVTLTCGSSTGAVTSGYYPNWVQQKPGQAPRGLIGGTKFLAPGTPARFSGSLLGGKAALTLSGVQPEDEAEYYCALWLANRWVFGGGTKLTVLGGGGSGGGGSGGGGSEVQLVESGGGLVQPGGSLKLSCAASGFTFNKYAMNWVRQAPGKGLEWVARIRSKYNNYATYYADSVKDRFTISRDDSKNTAYLQMNNLKTEDTAVYYCVRHGNFGNSYISYWAYWGQGTLVTVSS

SEQ ID NO: 77 - protein, 249 aa, synthetic construct
QTVVTQEPSLTVSPGGTVTLTCGSSTGTVTSGYYPNWVQQKPGQAPRGLIGGTKFLAPGTPARFSGSLLGGKAALTLSGVQPEDEAEYYCALWLSNRWVFGGGTKLTVLGGGGSGGGGSGGGGSEVQLVESGGGLVQPGGSLKLSCAASGFTFNKYAMNWVRQAPGKGLEWVARIRSKYNNYATYYADSVKDRFTISRDDSKNTAYLQMNNLKTEDTAVYYCVRHGNFGNSGISYWAYWGQGTLVTVSS

SEQ ID NO: 78 - protein, 249 aa, synthetic construct
QTVVTQEPSLTVSPGGTVTLTCGSSTGAVTSGYYPNWVQQKPGQAPRGLIGGTKFLAPGTPARFSGSLLGGKAALTLSGVQPEDEAEYYCALWYSNRWVFGGGTKLTVLGGGGSGGGGSGGGGSEVQLVESGGGLVQPGGSLKLSCAASGFTFNKYAMNWVRQAPGKGLEWVARIRSKYNNYATYYADSVKDRFTISRDDSKNTAYLQMNNLKTEDTAVYYCVRHGNFGTSYISYWAYWGQGTLVTVSS

SEQ ID NO: 79 - protein, 249 aa, synthetic construct
QTVVTQEPSLTVSPGGTVTLTCGSSTGAVTSGYYPNWVQQKPGQAPRGLIGGTKFLAPGTPARFSGSLLGGKAALTLSGVQPEDEAEYYCALWYSNRWVFGGGTKLTVLGGGGSGGGGSGGGGSEVQLVESGGGLVQPGGSLKLSCAASGFTFNKYAMNWVRQAPGKGLEWVARIRSKYNNYATYYADSVKDRFTISRDDSKNTAYLQMNNLKTEDTAVYYCVRHGNFGNTGISYWAYWGQGTLVTVSS

SEQ ID NO: 80 - protein, 249 aa, synthetic construct
QTVVTQEPSLTVSPGGTVTLTCGSSTGAVTSGYYPNWVQQKPGQAPRGLIGGTKFLAPGTPARFSGSLLGGKAALTLSGVQPEDEAEYYCALWYSGQWVFGGGTKLTVLGGGGSGGGGSGGGGSEVQLVESGGGLVQPGGSLKLSCAASGFTFNKYAMNWVRQAPGKGLEWVARIRSKYNNYATYYADSVKDRFTISRDDSKNTAYLQMNNLKTEDTAVYYCVRHGNFGNSYISYWAYWGQGTLVTVSS

SEQ ID NO: 81 - protein, 198 aa, synthetic construct
MQSGTRWRVLGLCLLSIGVWGQDGNEEMGSITQTPYQVSISGTTVILTCSQHLGSEAQWQHNGKNKEDSGDRLFLPEFSEMEQSGYYVCYPRGSNPEDASHHLYLKARVCENCMEMDVMAVATIVIVDICITLGLLLLVYYWSKNRKAKAKPVTRGAGAGGRQRGQNKERPPPVPNPDYEPIRKGQQDLYSGLNQRRI